European Patent Application EP 4 756 025 A1, published June 10, 2026. Title: DSRNA TARGETING MAPT AND PHARMACEUTICAL USE THEREOF. Applicant: TUOJIE BIOTECH (SHANGHAI) CO., LTD. The sequence listing filed with the application follows.

SEQUENCE LISTING (300 sequences)

SEQ ID NO: 1 - RNA, 19 nt, Synthetic Construct
  source 1..19: mol_type = other RNA; note = Unmodified sense strand of dsRNA
gggcggagatcgtgtacaa

SEQ ID NO: 2 - RNA, 19 nt, Synthetic Construct
  source 1..19: mol_type = other RNA; note = Unmodified sense strand of dsRNA
ggcggaggaaataaaaaga

SEQ ID NO: 3 - RNA, 19 nt, Synthetic Construct
  source 1..19: mol_type = other RNA; note = Unmodified sense strand of dsRNA
gggactggaagcgatgaca

SEQ ID NO: 4 - RNA, 19 nt, Synthetic Construct
  source 1..19: mol_type = other RNA; note = Unmodified sense strand of dsRNA
gactggaagcgatgacaaa

SEQ ID NO: 5 - RNA, 19 nt, Synthetic Construct
  source 1..19: mol_type = other RNA; note = Unmodified sense strand of dsRNA
gcggaggaaataaaaagat

SEQ ID NO: 6 - RNA, 19 nt, Synthetic Construct
  source 1..19: mol_type = other RNA; note = Unmodified sense strand of dsRNA
aaaaagattgaaacccaca

SEQ ID NO: 7 - RNA, 19 nt, Synthetic Construct
  source 1..19: mol_type = other RNA; note = Unmodified sense strand of dsRNA
gctacaccatgcaccaaga

SEQ ID NO: 8 - RNA, 19 nt, Synthetic Construct
  source 1..19: mol_type = other RNA; note = Unmodified sense strand of dsRNA
ccagacctgaagaatgtca

SEQ ID NO: 9 - RNA, 19 nt, Synthetic Construct
  source 1..19: mol_type = other RNA; note = Unmodified sense strand of dsRNA
cagacctgaagaatgtcaa

SEQ ID NO: 10 - RNA, 19 nt, Synthetic Construct
  source 1..19: mol_type = other RNA; note = Unmodified sense strand of dsRNA
ctgaagaatgtcaagtcca

SEQ ID NO: 11 - RNA, 21 nt, Synthetic Construct
  source 1..21: mol_type = other RNA; note = Unmodified antisense strand of dsRNA
ttgtacacgatctccgccccg

SEQ ID NO: 12 - RNA, 21 nt, Synthetic Construct
  source 1..21: mol_type = other RNA; note = Unmodified antisense strand of dsRNA
tctttttatttcctccgccag

SEQ ID NO: 13 - RNA, 21 nt, Synthetic Construct
  source 1..21: mol_type = other RNA; note = Unmodified antisense strand of dsRNA
tgtcatcgcttccagtcccgt

SEQ ID NO: 14 - RNA, 21 nt, Synthetic Construct
  source 1..21: mol_type = other RNA; note = Unmodified antisense strand of dsRNA
tttgtcatcgcttccagtccc

SEQ ID NO: 15 - RNA, 21 nt, Synthetic Construct
  source 1..21: mol_type = other RNA; note = Unmodified antisense strand of dsRNA
atctttttatttcctccgcca

SEQ ID NO: 16 - RNA, 21 nt, Synthetic Construct
  source 1..21: mol_type = other RNA; note = Unmodified antisense strand of dsRNA
tgtgggtttcaatctttttat

SEQ ID NO: 17 - RNA, 21 nt, Synthetic Construct
  source 1..21: mol_type = other RNA; note = Unmodified antisense strand of dsRNA
tcttggtgcatggtgtagccc

SEQ ID NO: 18 - RNA, 21 nt, Synthetic Construct
  source 1..21: mol_type = other RNA; note = Unmodified antisense strand of dsRNA
tgacattcttcaggtctggca

SEQ ID NO: 19 - RNA, 21 nt, Synthetic Construct
  source 1..21: mol_type = other RNA; note = Unmodified antisense strand of dsRNA
ttgacattcttcaggtctggc

SEQ ID NO: 20 - RNA, 21 nt, Synthetic Construct
  source 1..21: mol_type = other RNA; note = Unmodified antisense strand of dsRNA
tggacttgacattcttcaggt

SEQ ID NO: 21 - RNA, 19 nt, Synthetic Construct
  source 1..19: mol_type = other RNA; note = Unmodified sense strand of dsRNA
ccaccaggattccagcaaa

SEQ ID NO: 22 - RNA, 19 nt, Synthetic Construct
  source 1..19: mol_type = other RNA; note = Unmodified sense strand of dsRNA
cgatgacaaaaaagccaaa

SEQ ID NO: 23 - RNA, 19 nt, Synthetic Construct
  source 1..19: mol_type = other RNA; note = Unmodified sense strand of dsRNA
ggacacgtctccacggcat

SEQ ID NO: 24 - RNA, 19 nt, Synthetic Construct
  source 1..19: mol_type = other RNA; note = Unmodified sense strand of dsRNA
gggggacaggaaagatcaa

SEQ ID NO: 25 - RNA, 19 nt, Synthetic Construct
  source 1..19: mol_type = other RNA; note = Unmodified sense strand of dsRNA
cctggaagacgaagctgct

SEQ ID NO: 26 - RNA, 19 nt, Synthetic Construct
  source 1..19: mol_type = other RNA; note = Unmodified sense strand of dsRNA
ggactggaagcgatgacaa

SEQ ID NO: 27 - RNA, 19 nt, Synthetic Construct
  source 1..19: mol_type = other RNA; note = Unmodified sense strand of dsRNA
ctggaagcgatgacaaaaa

SEQ ID NO: 28 - RNA, 19 nt, Synthetic Construct
  source 1..19: mol_type = other RNA; note = Unmodified sense strand of dsRNA
ggaagcgatgacaaaaaaa

SEQ ID NO: 29 - RNA, 19 nt, Synthetic Construct
  source 1..19: mol_type = other RNA; note = Unmodified sense strand of dsRNA
ccatgccagacctgaagaa

SEQ ID NO: 30 - RNA, 19 nt, Synthetic Construct
  source 1..19: mol_type = other RNA; note = Unmodified sense strand of dsRNA
aaaagattgaaacccacaa

SEQ ID NO: 31 - RNA, 19 nt, Synthetic Construct
  source 1..19: mol_type = other RNA; note = Unmodified sense strand of dsRNA
gcgagaacgccaaagccaa

SEQ ID NO: 32 - RNA, 19 nt, Synthetic Construct
  source 1..19: mol_type = other RNA; note = Unmodified sense strand of dsRNA
cctccatgtagaagaggga

SEQ ID NO: 33 - RNA, 19 nt, Synthetic Construct
  source 1..19: mol_type = other RNA; note = Unmodified sense strand of dsRNA
ccatgtagaagagggagaa

SEQ ID NO: 34 - RNA, 19 nt, Synthetic Construct
  source 1..19: mol_type = other RNA; note = Unmodified sense strand of dsRNA
gtgtgttcgtggagccaca

SEQ ID NO: 35 - RNA, 19 nt, Synthetic Construct
  source 1..19: mol_type = other RNA; note = Unmodified sense strand of dsRNA
gggagacgtccacccgttt

SEQ ID NO: 36 - RNA, 19 nt, Synthetic Construct
  source 1..19: mol_type = other RNA; note = Unmodified sense strand of dsRNA
caccaggattccagcaaaa

SEQ ID NO: 37 - RNA, 19 nt, Synthetic Construct
  source 1..19: mol_type = other RNA; note = Unmodified sense strand of dsRNA
cgcaccccgtcccttccaa

SEQ ID NO: 38 - RNA, 19 nt, Synthetic Construct
  source 1..19: mol_type = other RNA; note = Unmodified sense strand of dsRNA
gcctcttgggagacgtcca

SEQ ID NO: 39 - RNA, 19 nt, Synthetic Construct
  source 1..19: mol_type = other RNA; note = Unmodified sense strand of dsRNA
gcctatacccctcatcaca

SEQ ID NO: 40 - RNA, 19 nt, Synthetic Construct
  source 1..19: mol_type = other RNA; note = Unmodified sense strand of dsRNA
gcacaagagtgggacccca

SEQ ID NO: 41 - RNA, 19 nt, Synthetic Construct
  source 1..19: mol_type = other RNA; note = Unmodified sense strand of dsRNA
ccccagcctggaagacgaa

SEQ ID NO: 42 - RNA, 19 nt, Synthetic Construct
  source 1..19: mol_type = other RNA; note = Unmodified sense strand of dsRNA
gcgatgacaaaaaagccaa

SEQ ID NO: 43 - RNA, 19 nt, Synthetic Construct
  source 1..19: mol_type = other RNA; note = Unmodified sense strand of dsRNA
gccaccaggattccagcaa

SEQ ID NO: 44 - RNA, 19 nt, Synthetic Construct
  source 1..19: mol_type = other RNA; note = Unmodified sense strand of dsRNA
cctggcggaggaaataaaa

SEQ ID NO: 45 - RNA, 19 nt, Synthetic Construct
  source 1..19: mol_type = other RNA; note = Unmodified sense strand of dsRNA
ctggcggaggaaataaaaa

SEQ ID NO: 46 - RNA, 19 nt, Synthetic Construct
  source 1..19: mol_type = other RNA; note = Unmodified sense strand of dsRNA
gcggaggaaataaaaagaa

SEQ ID NO: 47 - RNA, 19 nt, Synthetic Construct
  source 1..19: mol_type = other RNA; note = Unmodified sense strand of dsRNA
agctgaccttccgcgagaa

SEQ ID NO: 48 - RNA, 19 nt, Synthetic Construct
  source 1..19: mol_type = other RNA; note = Unmodified sense strand of dsRNA
ccttccgcgagaacgccaa

SEQ ID NO: 49 - RNA, 19 nt, Synthetic Construct
  source 1..19: mol_type = other RNA; note = Unmodified sense strand of dsRNA
cttccgcgagaacgccaaa

SEQ ID NO: 50 - RNA, 19 nt, Synthetic Construct
  source 1..19: mol_type = other RNA; note = Unmodified sense strand of dsRNA
cgcgagaacgccaaagcca

SEQ ID NO: 51 - RNA, 19 nt, Synthetic Construct
  source 1..19: mol_type = other RNA; note = Unmodified sense strand of dsRNA
ggggtgtcacagaggcagt

SEQ ID NO: 52 - RNA, 19 nt, Synthetic Construct
  source 1..19: mol_type = other RNA; note = Unmodified sense strand of dsRNA
gacgtccacccgtttccaa

SEQ ID NO: 53 - RNA, 19 nt, Synthetic Construct
  source 1..19: mol_type = other RNA; note = Unmodified sense strand of dsRNA
gggcactgctcagctgtga

SEQ ID NO: 54 - RNA, 19 nt, Synthetic Construct
  source 1..19: mol_type = other RNA; note = Unmodified sense strand of dsRNA
gctcagctccacatgcata

SEQ ID NO: 55 - RNA, 19 nt, Synthetic Construct
  source 1..19: mol_type = other RNA; note = Unmodified sense strand of dsRNA
ggaacacacccccttggaa

SEQ ID NO: 56 - RNA, 19 nt, Synthetic Construct
  source 1..19: mol_type = other RNA; note = Unmodified sense strand of dsRNA
ctgagaacctgaagcacca

SEQ ID NO: 57 - RNA, 19 nt, Synthetic Construct
  source 1..19: mol_type = other RNA; note = Unmodified sense strand of dsRNA
ggaactgctgccatgattt

SEQ ID NO: 58 - RNA, 19 nt, Synthetic Construct
  source 1..19: mol_type = other RNA; note = Unmodified sense strand of dsRNA
ctgggaccctcaccacgaa

SEQ ID NO: 59 - RNA, 19 nt, Synthetic Construct
  source 1..19: mol_type = other RNA; note = Unmodified sense strand of dsRNA
gccagaagggccaggccaa

SEQ ID NO: 60 - RNA, 19 nt, Synthetic Construct
  source 1..19: mol_type = other RNA; note = Unmodified sense strand of dsRNA
ggccaacgccaccaggatt

SEQ ID NO: 61 - RNA, 19 nt, Synthetic Construct
  source 1..19: mol_type = other RNA; note = Unmodified sense strand of dsRNA
aaaacatggccacatccaa

SEQ ID NO: 62 - RNA, 19 nt, Synthetic Construct
  source 1..19: mol_type = other RNA; note = Unmodified sense strand of dsRNA
gaactgctgccatgatttt

SEQ ID NO: 63 - RNA, 19 nt, Synthetic Construct
  source 1..19: mol_type = other RNA; note = Unmodified sense strand of dsRNA
ccttctcagtaatgaccct

SEQ ID NO: 64 - RNA, 19 nt, Synthetic Construct
  source 1..19: mol_type = other RNA; note = Unmodified sense strand of dsRNA
catccaactgggaccctca

SEQ ID NO: 65 - RNA, 19 nt, Synthetic Construct
  source 1..19: mol_type = other RNA; note = Unmodified sense strand of dsRNA
ccctcaccacgaatctcat

SEQ ID NO: 66 - RNA, 19 nt, Synthetic Construct
  source 1..19: mol_type = other RNA; note = Unmodified sense strand of dsRNA
ccgtcacagatgtgagcca

SEQ ID NO: 67 - RNA, 19 nt, Synthetic Construct
  source 1..19: mol_type = other RNA; note = Unmodified sense strand of dsRNA
gaacacacccccttggaaa

SEQ ID NO: 68 - RNA, 19 nt, Synthetic Construct
  source 1..19: mol_type = other RNA; note = Unmodified sense strand of dsRNA
ggcagtggtccgtactcca

SEQ ID NO: 69 - RNA, 19 nt, Synthetic Construct
  source 1..19: mol_type = other RNA; note = Unmodified sense strand of dsRNA
cgaagattgggtccctgga

SEQ ID NO: 70 - RNA, 19 nt, Synthetic Construct
  source 1..19: mol_type = other RNA; note = Unmodified sense strand of dsRNA
ggttggaactgctgccata

SEQ ID NO: 71 - RNA, 19 nt, Synthetic Construct
  source 1..19: mol_type = other RNA; note = Unmodified sense strand of dsRNA
ggtacctactccatactga

SEQ ID NO: 72 - RNA, 19 nt, Synthetic Construct
  source 1..19: mol_type = other RNA; note = Unmodified sense strand of dsRNA
agattgggtccctggacaa

SEQ ID NO: 73 - RNA, 19 nt, Synthetic Construct
  source 1..19: mol_type = other RNA; note = Unmodified sense strand of dsRNA
gggtccctggacaatatca

SEQ ID NO: 74 - RNA, 19 nt, Synthetic Construct
  source 1..19: mol_type = other RNA; note = Unmodified sense strand of dsRNA
agaaggagaggctctgaaa

SEQ ID NO: 75 - RNA, 19 nt, Synthetic Construct
  source 1..19: mol_type = other RNA; note = Unmodified sense strand of dsRNA
ccctgttgtgggggtgtca

SEQ ID NO: 76 - RNA, 19 nt, Synthetic Construct
  source 1..19: mol_type = other RNA; note = Unmodified sense strand of dsRNA
ctgttgtgggggtgtcaca

SEQ ID NO: 77 - RNA, 21 nt, Synthetic Construct
  source 1..21: mol_type = other RNA; note = Unmodified sense strand of dsRNA
gagatcgtgtacaagtcgcca

SEQ ID NO: 78 - RNA, 18 nt, Synthetic Construct
  source 1..18: mol_type = other RNA; note = Unmodified sense strand of dsRNA
ggcggagatcgtgtacaa

SEQ ID NO: 79 - RNA, 21 nt, Synthetic Construct
  source 1..21: mol_type = other RNA; note = Unmodified antisense strand of dsRNA
tttgctggaatcctggtggcg

SEQ ID NO: 80 - RNA, 21 nt, Synthetic Construct
  source 1..21: mol_type = other RNA; note = Unmodified antisense strand of dsRNA
tttggcttttttgtcatcgct

SEQ ID NO: 81 - RNA, 21 nt, Synthetic Construct
  source 1..21: mol_type = other RNA; note = Unmodified antisense strand of dsRNA
atgccgtggagacgtgtcccc

SEQ ID NO: 82 - RNA, 21 nt, Synthetic Construct
  source 1..21: mol_type = other RNA; note = Unmodified antisense strand of dsRNA
ttgatctttcctgtcccccaa

SEQ ID NO: 83 - RNA, 21 nt, Synthetic Construct
  source 1..21: mol_type = other RNA; note = Unmodified antisense strand of dsRNA
agcagcttcgtcttccaggct

SEQ ID NO: 84 - RNA, 21 nt, Synthetic Construct
  source 1..21: mol_type = other RNA; note = Unmodified antisense strand of dsRNA
ttgtcatcgcttccagtcccg

SEQ ID NO: 85 - RNA, 21 nt, Synthetic Construct
  source 1..21: mol_type = other RNA; note = Unmodified antisense strand of dsRNA
tttttgtcatcgcttccagtc

SEQ ID NO: 86 - RNA, 21 nt, Synthetic Construct
  source 1..21: mol_type = other RNA; note = Unmodified antisense strand of dsRNA
tttttttgtcatcgcttccag

SEQ ID NO: 87 - RNA, 21 nt, Synthetic Construct
  source 1..21: mol_type = other RNA; note = Unmodified antisense strand of dsRNA
ttcttcaggtctggcatgggc

SEQ ID NO: 88 - RNA, 21 nt, Synthetic Construct
  source 1..21: mol_type = other RNA; note = Unmodified antisense strand of dsRNA
ttgtgggtttcaatcttttta

SEQ ID NO: 89 - RNA, 21 nt, Synthetic Construct
  source 1..21: mol_type = other RNA; note = Unmodified antisense strand of dsRNA
ttggctttggcgttctcgcgg

SEQ ID NO: 90 - RNA, 21 nt, Synthetic Construct
  source 1..21: mol_type = other RNA; note = Unmodified antisense strand of dsRNA
tccctcttctacatggagggg

SEQ ID NO: 91 - RNA, 21 nt, Synthetic Construct
  source 1..21: mol_type = other RNA; note = Unmodified antisense strand of dsRNA
ttctccctcttctacatggag

SEQ ID NO: 92 - RNA, 21 nt, Synthetic Construct
  source 1..21: mol_type = other RNA; note = Unmodified antisense strand of dsRNA
tgtggctccacgaacacacca

SEQ ID NO: 93 - RNA, 21 nt, Synthetic Construct
  source 1..21: mol_type = other RNA; note = Unmodified antisense strand of dsRNA
aaacgggtggacgtctcccaa

SEQ ID NO: 94 - RNA, 21 nt, Synthetic Construct
  source 1..21: mol_type = other RNA; note = Unmodified antisense strand of dsRNA
ttttgctggaatcctggtggc

SEQ ID NO: 95 - RNA, 21 nt, Synthetic Construct
  source 1..21: mol_type = other RNA; note = Unmodified antisense strand of dsRNA
ttggaagggacggggtgcggg

SEQ ID NO: 96 - RNA, 21 nt, Synthetic Construct
  source 1..21: mol_type = other RNA; note = Unmodified antisense strand of dsRNA
tggacgtctcccaagaggcac

SEQ ID NO: 97 - RNA, 21 nt, Synthetic Construct
  source 1..21: mol_type = other RNA; note = Unmodified antisense strand of dsRNA
tgtgatgaggggtataggcag

SEQ ID NO: 98 - RNA, 21 nt, Synthetic Construct
  source 1..21: mol_type = other RNA; note = Unmodified antisense strand of dsRNA
tggggtcccactcttgtgcct

SEQ ID NO: 99 - RNA, 21 nt, Synthetic Construct
  source 1..21: mol_type = other RNA; note = Unmodified antisense strand of dsRNA
ttcgtcttccaggctgggggt

SEQ ID NO: 100 - RNA, 21 nt, Synthetic Construct
  source 1..21: mol_type = other RNA; note = Unmodified antisense strand of dsRNA
ttggcttttttgtcatcgctt

SEQ ID NO: 101 - RNA, 21 nt, Synthetic Construct
  source 1..21: mol_type = other RNA; note = Unmodified antisense strand of dsRNA
ttgctggaatcctggtggcgt

SEQ ID NO: 102 - RNA, 21 nt, Synthetic Construct
  source 1..21: mol_type = other RNA; note = Unmodified antisense strand of dsRNA
ttttatttcctccgccaggga

SEQ ID NO: 103 - RNA, 21 nt, Synthetic Construct
  source 1..21: mol_type = other RNA; note = Unmodified antisense strand of dsRNA
tttttatttcctccgccaggg

SEQ ID NO: 104 - RNA, 21 nt, Synthetic Construct
  source 1..21: mol_type = other RNA; note = Unmodified antisense strand of dsRNA
ttctttttatttcctccgcca

SEQ ID NO: 105 - RNA, 21 nt, Synthetic Construct
  source 1..21: mol_type = other RNA; note = Unmodified antisense strand of dsRNA
ttctcgcggaaggtcagcttg

SEQ ID NO: 106 - RNA, 21 nt, Synthetic Construct
  source 1..21: mol_type = other RNA; note = Unmodified antisense strand of dsRNA
ttggcgttctcgcggaaggtc

SEQ ID NO: 107 - RNA, 21 nt, Synthetic Construct
  source 1..21: mol_type = other RNA; note = Unmodified antisense strand of dsRNA
tttggcgttctcgcggaaggt

SEQ ID NO: 108 - RNA, 21 nt, Synthetic Construct
  source 1..21: mol_type = other RNA; note = Unmodified antisense strand of dsRNA
tggctttggcgttctcgcgga

SEQ ID NO: 109 - RNA, 21 nt, Synthetic Construct
  source 1..21: mol_type = other RNA; note = Unmodified antisense strand of dsRNA
actgcctctgtgacaccccca

SEQ ID NO: 110 - RNA, 21 nt, Synthetic Construct
  source 1..21: mol_type = other RNA; note = Unmodified antisense strand of dsRNA
ttggaaacgggtggacgtctc

SEQ ID NO: 111 - RNA, 21 nt, Synthetic Construct
  source 1..21: mol_type = other RNA; note = Unmodified antisense strand of dsRNA
tcacagctgagcagtgccctg

SEQ ID NO: 112 - RNA, 21 nt, Synthetic Construct
  source 1..21: mol_type = other RNA; note = Unmodified antisense strand of dsRNA
tatgcatgtggagctgagcag

SEQ ID NO: 113 - RNA, 21 nt, Synthetic Construct
  source 1..21: mol_type = other RNA; note = Unmodified antisense strand of dsRNA
ttccaagggggtgtgttcccc

SEQ ID NO: 114 - RNA, 21 nt, Synthetic Construct
  source 1..21: mol_type = other RNA; note = Unmodified antisense strand of dsRNA
tggtgcttcaggttctcagtg

SEQ ID NO: 115 - RNA, 21 nt, Synthetic Construct
  source 1..21: mol_type = other RNA; note = Unmodified antisense strand of dsRNA
aaatcatggcagcagttccaa

SEQ ID NO: 116 - RNA, 21 nt, Synthetic Construct
  source 1..21: mol_type = other RNA; note = Unmodified antisense strand of dsRNA
ttcgtggtgagggtcccagtt

SEQ ID NO: 117 - RNA, 21 nt, Synthetic Construct
  source 1..21: mol_type = other RNA; note = Unmodified antisense strand of dsRNA
ttggcctggcccttctggcct

SEQ ID NO: 118 - RNA, 21 nt, Synthetic Construct
  source 1..21: mol_type = other RNA; note = Unmodified antisense strand of dsRNA
aatcctggtggcgttggcctg

SEQ ID NO: 119 - RNA, 21 nt, Synthetic Construct
  source 1..21: mol_type = other RNA; note = Unmodified antisense strand of dsRNA
ttggatgtggccatgtttttg

SEQ ID NO: 120 - RNA, 21 nt, Synthetic Construct
  source 1..21: mol_type = other RNA; note = Unmodified antisense strand of dsRNA
aaaatcatggcagcagttcca

SEQ ID NO: 121 - RNA, 21 nt, Synthetic Construct
  source 1..21: mol_type = other RNA; note = Unmodified antisense strand of dsRNA
agggtcattactgagaagggg

SEQ ID NO: 122 - RNA, 21 nt, Synthetic Construct
  source 1..21: mol_type = other RNA; note = Unmodified antisense strand of dsRNA
tgagggtcccagttggatgag

SEQ ID NO: 123 - RNA, 21 nt, Synthetic Construct
  source 1..21: mol_type = other RNA; note = Unmodified antisense strand of dsRNA
atgagattcgtggtgagggtc

SEQ ID NO: 124 - RNA, 21 nt, Synthetic Construct
  source 1..21: mol_type = other RNA; note = Unmodified antisense strand of dsRNA
tggctcacatctgtgacggga

SEQ ID NO: 125 - RNA, 21 nt, Synthetic Construct
  source 1..21: mol_type = other RNA; note = Unmodified antisense strand of dsRNA
tttccaagggggtgtgttccc

SEQ ID NO: 126 - RNA, 21 nt, Synthetic Construct
  source 1..21: mol_type = other RNA; note = Unmodified antisense strand of dsRNA
tggagtacggaccactgccac

SEQ ID NO: 127 - RNA, 21 nt, Synthetic Construct
  source 1..21: mol_type = other RNA; note = Unmodified antisense strand of dsRNA
tccagggacccaatcttcgac

SEQ ID NO: 128 - RNA, 21 nt, Synthetic Construct
  source 1..21: mol_type = other RNA; note = Unmodified antisense strand of dsRNA
tatggcagcagttccaacctt

SEQ ID NO: 129 - RNA, 21 nt, Synthetic Construct
  source 1..21: mol_type = other RNA; note = Unmodified antisense strand of dsRNA
tcagtatggagtaggtacctc

SEQ ID NO: 130 - RNA, 21 nt, Synthetic Construct
  source 1..21: mol_type = other RNA; note = Unmodified antisense strand of dsRNA
ttgtccagggacccaatcttc

SEQ ID NO: 131 - RNA, 21 nt, Synthetic Construct
  source 1..21: mol_type = other RNA; note = Unmodified antisense strand of dsRNA
tgatattgtccagggacccaa

SEQ ID NO: 132 - RNA, 21 nt, Synthetic Construct
  source 1..21: mol_type = other RNA; note = Unmodified antisense strand of dsRNA
tttcagagcctctccttctcc

SEQ ID NO: 133 - RNA, 21 nt, Synthetic Construct
  source 1..21: mol_type = other RNA; note = Unmodified antisense strand of dsRNA
tgacacccccacaacagggcc

SEQ ID NO: 134 - RNA, 21 nt, Synthetic Construct
  source 1..21: mol_type = other RNA; note = Unmodified antisense strand of dsRNA
tgtgacacccccacaacaggg

SEQ ID NO: 135 - RNA, 23 nt, Synthetic Construct
  source 1..23: mol_type = other RNA; note = Unmodified antisense strand of dsRNA
tggcgacttgtacacgatctccg

SEQ ID NO: 136 - RNA, 18 nt, Synthetic Construct
  source 1..18: mol_type = other RNA; note = Unmodified antisense strand of dsRNA
ttgtacacgatctccgcc

SEQ ID NO: 137 - RNA, 19 nt, Synthetic Construct
  source 1..19: mol_type = other RNA; note = Modified sense strand of dsRNA
  modified_base 1..19: mod_base = OTHER; note = having modifications as shown in Table 3 of the specification
ggcggaggaaataaaaaga

SEQ ID NO: 138 - RNA, 19 nt, Synthetic Construct
  source 1..19: mol_type = other RNA; note = modified sense strand of dsRNA; note (original language) = Modified sense strand of dsRNA
  modified_base 1..19: mod_base = OTHER; note = having modifications as shown in Table 3 of the specification
gggactggaagcgatgaca

SEQ ID NO: 139 - RNA, 19 nt, Synthetic Construct
  source 1..19: mol_type = other RNA; note = modified sense strand of dsRNA; note (original language) = Modified sense strand of dsRNA
  modified_base 1..19: mod_base = OTHER; note = having modifications as shown in Table 3 of the specification
gactggaagcgatgacaaa

SEQ ID NO: 140 - RNA, 19 nt, Synthetic Construct
  source 1..19: mol_type = other RNA; note = modified sense strand of dsRNA; note (original language) = Modified sense strand of dsRNA
  modified_base 1..19: mod_base = OTHER; note = having modifications as shown in Table 3 of the specification
gcggaggaaataaaaagaa

SEQ ID NO: 141 - RNA, 19 nt, Synthetic Construct
  source 1..19: mol_type = other RNA; note = modified sense strand of dsRNA; note (original language) = Modified sense strand of dsRNA
  modified_base 1..19: mod_base = OTHER; note = having modifications as shown in Table 3 of the specification
aaaaagattgaaacccaca

SEQ ID NO: 142 - RNA, 19 nt, Synthetic Construct
  source 1..19: mol_type = other RNA; note = modified sense strand of dsRNA; note (original language) = Modified sense strand of dsRNA
  modified_base 1..19: mod_base = OTHER; note = having modifications as shown in Table 3 of the specification
gctacaccatgcaccaaga

SEQ ID NO: 143 - RNA, 19 nt, Synthetic Construct
  source 1..19: mol_type = other RNA; note = modified sense strand of dsRNA; note (original language) = Modified sense strand of dsRNA
  modified_base 1..19: mod_base = OTHER; note = having modifications as shown in Table 3 of the specification
ccagacctgaagaatgtca

SEQ ID NO: 144 - RNA, 19 nt, Synthetic Construct
  source 1..19: mol_type = other RNA; note = modified sense strand of dsRNA; note (original language) = Modified sense strand of dsRNA
  modified_base 1..19: mod_base = OTHER; note = having modifications as shown in Table 3 of the specification
gggcggagatcgtgtacaa

SEQ ID NO: 145 - RNA, 19 nt, Synthetic Construct
  source 1..19: mol_type = other RNA; note = modified sense strand of dsRNA; note (original language) = Modified sense strand of dsRNA
  modified_base 1..19: mod_base = OTHER; note = having modifications as shown in Table 3 of the specification
cagacctgaagaatgtcaa

SEQ ID NO: 146 - RNA, 19 nt, Synthetic Construct
  source 1..19: mol_type = other RNA; note = modified sense strand of dsRNA; note (original language) = Modified sense strand of dsRNA
  modified_base 1..19: mod_base = OTHER; note = having modifications as shown in Table 3 of the specification
ctgaagaatgtcaagtcca

SEQ ID NO: 147 - RNA, 19 nt, Synthetic Construct
  source 1..19: mol_type = other RNA; note = modified sense strand of dsRNA; note (original language) = Modified sense strand of dsRNA
  modified_base 1..19: mod_base = OTHER; note = having modifications as shown in Table 3 of the specification
ccaccaggattccagcaaa

SEQ ID NO: 148 - RNA, 19 nt, Synthetic Construct
  source 1..19: mol_type = other RNA; note = modified sense strand of dsRNA; note (original language) = Modified sense strand of dsRNA
  modified_base 1..19: mod_base = OTHER; note = having modifications as shown in Table 3 of the specification
cgatgacaaaaaagccaaa

SEQ ID NO: 149 - RNA, 19 nt, Synthetic Construct
  source 1..19: mol_type = other RNA; note = modified sense strand of dsRNA; note (original language) = Modified sense strand of dsRNA
  modified_base 1..19: mod_base = OTHER; note = having modifications as shown in Table 3 of the specification
ggacacgtctccacggcaa

SEQ ID NO: 150 - RNA, 19 nt, Synthetic Construct
  source 1..19: mol_type = other RNA; note = modified sense strand of dsRNA; note (original language) = Modified sense strand of dsRNA
  modified_base 1..19: mod_base = OTHER; note = having modifications as shown in Table 3 of the specification
gggggacaggaaagatcaa

SEQ ID NO: 151 - RNA, 19 nt, Synthetic Construct
  source 1..19: mol_type = other RNA; note = modified sense strand of dsRNA; note (original language) = Modified sense strand of dsRNA
  modified_base 1..19: mod_base = OTHER; note = having modifications as shown in Table 3 of the specification
cctggaagacgaagctgca

SEQ ID NO: 152 - RNA, 19 nt, Synthetic Construct
  source 1..19: mol_type = other RNA; note = modified sense strand of dsRNA; note (original language) = Modified sense strand of dsRNA
  modified_base 1..19: mod_base = OTHER; note = having modifications as shown in Table 3 of the specification
ggactggaagcgatgacaa

SEQ ID NO: 153 - RNA, 19 nt, Synthetic Construct
  source 1..19: mol_type = other RNA; note = modified sense strand of dsRNA; note (original language) = Modified sense strand of dsRNA
  modified_base 1..19: mod_base = OTHER; note = having modifications as shown in Table 3 of the specification
ctggaagcgatgacaaaaa

SEQ ID NO: 154 - RNA, 19 nt, Synthetic Construct
  source 1..19: mol_type = other RNA; note = modified sense strand of dsRNA; note (original language) = Modified sense strand of dsRNA
  modified_base 1..19: mod_base = OTHER; note = having modifications as shown in Table 3 of the specification
ggaagcgatgacaaaaaaa

SEQ ID NO: 155 - RNA, 19 nt, Synthetic Construct
  source 1..19: mol_type = other RNA; note = modified sense strand of dsRNA; note (original language) = Modified sense strand of dsRNA
  modified_base 1..19: mod_base = OTHER; note = having modifications as shown in Table 3 of the specification
ccatgccagacctgaagaa

SEQ ID NO: 156 - RNA, 19 nt, Synthetic Construct
  source 1..19: mol_type = other RNA; note = modified sense strand of dsRNA; note (original language) = Modified sense strand of dsRNA
  modified_base 1..19: mod_base = OTHER; note = having modifications as shown in Table 3 of the specification
aaaagattgaaacccacaa

SEQ ID NO: 157 - RNA, 19 nt, Synthetic Construct
  source 1..19: mol_type = other RNA; note = modified sense strand of dsRNA; note (original language) = Modified sense strand of dsRNA
  modified_base 1..19: mod_base = OTHER; note = having modifications as shown in Table 3 of the specification
gcgagaacgccaaagccaa

SEQ ID NO: 158 - RNA, 19 nt, Synthetic Construct
  source 1..19: mol_type = other RNA; note = modified sense strand of dsRNA; note (original language) = Modified sense strand of dsRNA
  modified_base 1..19: mod_base = OTHER; note = having modifications as shown in Table 3 of the specification
cctccatgtagaagaggga

SEQ ID NO: 159 - RNA, 19 nt, Synthetic Construct
  source 1..19: mol_type = other RNA; note = modified sense strand of dsRNA; note (original language) = Modified sense strand of dsRNA
  modified_base 1..19: mod_base = OTHER; note = having modifications as shown in Table 3 of the specification
ccatgtagaagagggagaa

SEQ ID NO: 160 - RNA, 19 nt, Synthetic Construct
  source 1..19: mol_type = other RNA; note = modified sense strand of dsRNA; note (original language) = Modified sense strand of dsRNA
  modified_base 1..19: mod_base = OTHER; note = having modifications as shown in Table 3 of the specification
gtgtgttcgtggagccaca

SEQ ID NO: 161 - RNA, 19 nt, Synthetic Construct
  source 1..19: mol_type = other RNA; note = modified sense strand of dsRNA; note (original language) = Modified sense strand of dsRNA
  modified_base 1..19: mod_base = OTHER; note = having modifications as shown in Table 3 of the specification
gggagacgtccacccgtta

SEQ ID NO: 162 - RNA, 19 nt, Synthetic Construct
  source 1..19: mol_type = other RNA; note = modified sense strand of dsRNA; note (original language) = Modified sense strand of dsRNA
  modified_base 1..19: mod_base = OTHER; note = having modifications as shown in Table 3 of the specification
caccaggattccagcaaaa

SEQ ID NO: 163 - RNA, 19 nt, Synthetic Construct
  source 1..19: mol_type = other RNA; note = modified sense strand of dsRNA; note (original language) = Modified sense strand of dsRNA
  modified_base 1..19: mod_base = OTHER; note = having modifications as shown in Table 3 of the specification
cgcaccccgtcccttccaa

SEQ ID NO: 164 - RNA, 19 nt, Synthetic Construct
  source 1..19: mol_type = other RNA; note = modified sense strand of dsRNA; note (original language) = Modified sense strand of dsRNA
  modified_base 1..19: mod_base = OTHER; note = having modifications as shown in Table 3 of the specification
gcctcttgggagacgtcca

SEQ ID NO: 165 - RNA, 19 nt, Synthetic Construct
  source 1..19: mol_type = other RNA; note = modified sense strand of dsRNA; note (original language) = Modified sense strand of dsRNA
  modified_base 1..19: mod_base = OTHER; note = having modifications as shown in Table 3 of the specification
gcctatacccctcatcaca

SEQ ID NO: 166 - RNA, 19 nt, Synthetic Construct
  source 1..19: mol_type = other RNA; note = modified sense strand of dsRNA; note (original language) = Modified sense strand of dsRNA
  modified_base 1..19: mod_base = OTHER; note = having modifications as shown in Table 3 of the specification
gcacaagagtgggacccca

SEQ ID NO: 167 - RNA, 19 nt, Synthetic Construct
  source 1..19: mol_type = other RNA; note = modified sense strand of dsRNA; note (original language) = Modified sense strand of dsRNA
  modified_base 1..19: mod_base = OTHER; note = having modifications as shown in Table 3 of the specification
ccccagcctggaagacgaa

SEQ ID NO: 168 - RNA, 19 nt, Synthetic Construct
  source 1..19: mol_type = other RNA; note = modified sense strand of dsRNA; note (original language) = Modified sense strand of dsRNA
  modified_base 1..19: mod_base = OTHER; note = having modifications as shown in Table 3 of the specification
gcgatgacaaaaaagccaa

SEQ ID NO: 169 - RNA, 19 nt, Synthetic Construct
  source 1..19: mol_type = other RNA; note = modified sense strand of dsRNA; note (original language) = Modified sense strand of dsRNA
  modified_base 1..19: mod_base = OTHER; note = having modifications as shown in Table 3 of the specification
gccaccaggattccagcaa

SEQ ID NO: 170 - RNA, 19 nt, Synthetic Construct
  source 1..19: mol_type = other RNA; note = modified sense strand of dsRNA; note (original language) = Modified sense strand of dsRNA
  modified_base 1..19: mod_base = OTHER; note = having modifications as shown in Table 3 of the specification
cctggcggaggaaataaaa

SEQ ID NO: 171 - RNA, 19 nt, Synthetic Construct
  source 1..19: mol_type = other RNA; note = modified sense strand of dsRNA; note (original language) = Modified sense strand of dsRNA
  modified_base 1..19: mod_base = OTHER; note = having modifications as shown in Table 3 of the specification
ctggcggaggaaataaaaa

SEQ ID NO: 172 - RNA, 19 nt, Synthetic Construct
  source 1..19: mol_type = other RNA; note = modified sense strand of dsRNA; note (original language) = Modified sense strand of dsRNA
  modified_base 1..19: mod_base = OTHER; note = having modifications as shown in Table 3 of the specification
agctgaccttccgcgagaa

SEQ ID NO: 173 - RNA, 19 nt, Synthetic Construct
  source 1..19: mol_type = other RNA; note = modified sense strand of dsRNA; note (original language) = Modified sense strand of dsRNA
  modified_base 1..19: mod_base = OTHER; note = having modifications as shown in Table 3 of the specification
ccttccgcgagaacgccaa

SEQ ID NO: 174 - RNA, 19 nt, Synthetic Construct
  source 1..19: mol_type = other RNA; note = modified sense strand of dsRNA; note (original language) = Modified sense strand of dsRNA
  modified_base 1..19: mod_base = OTHER; note = having modifications as shown in Table 3 of the specification
cttccgcgagaacgccaaa

SEQ ID NO: 175 - RNA, 19 nt, Synthetic Construct
  source 1..19: mol_type = other RNA; note = modified sense strand of dsRNA; note (original language) = Modified sense strand of dsRNA
  modified_base 1..19: mod_base = OTHER; note = having modifications as shown in Table 3 of the specification
cgcgagaacgccaaagcca

SEQ ID NO: 176 - RNA, 19 nt, Synthetic Construct
  source 1..19: mol_type = other RNA; note = modified sense strand of dsRNA; note (original language) = Modified sense strand of dsRNA
  modified_base 1..19: mod_base = OTHER; note = having modifications as shown in Table 3 of the specification
ggggtgtcacagaggcaga

SEQ ID NO: 177 - RNA, 19 nt, Synthetic Construct
  source 1..19: mol_type = other RNA; note = modified sense strand of dsRNA; note (original language) = Modified sense strand of dsRNA
  modified_base 1..19: mod_base = OTHER; note = having modifications as shown in Table 3 of the specification
gacgtccacccgtttccaa

SEQ ID NO: 178 - RNA, 19 nt, Synthetic Construct
  source 1..19: mol_type = other RNA; note = modified sense strand of dsRNA; note (original language) = Modified sense strand of dsRNA
  modified_base 1..19: mod_base = OTHER; note = having modifications as shown in Table 3 of the specification
gggcactgctcagctgtga

SEQ ID NO: 179 - RNA, 19 nt, Synthetic Construct
  source 1..19: mol_type = other RNA; note = modified sense strand of dsRNA; note (original language) = Modified sense strand of dsRNA
  modified_base 1..19: mod_base = OTHER; note = having modifications as shown in Table 3 of the specification
gctcagctccacatgcata

SEQ ID NO: 180 - RNA, 19 nt, Synthetic Construct
  source 1..19: mol_type = other RNA; note = modified sense strand of dsRNA; note (original language) = Modified sense strand of dsRNA
  modified_base 1..19: mod_base = OTHER; note = having modifications as shown in Table 3 of the specification
ggaacacacccccttggaa

SEQ ID NO: 181 - RNA, 19 nt, Synthetic Construct
  source 1..19: mol_type = other RNA; note = modified sense strand of dsRNA; note (original language) = Modified sense strand of dsRNA
  modified_base 1..19: mod_base = OTHER; note = having modifications as shown in Table 3 of the specification
ctgagaacctgaagcacca

SEQ ID NO: 182 - RNA, 19 nt, Synthetic Construct
  source 1..19: mol_type = other RNA; note = modified sense strand of dsRNA; note (original language) = Modified sense strand of dsRNA
  modified_base 1..19: mod_base = OTHER; note = having modifications as shown in Table 3 of the specification
ggaactgctgccatgatta

SEQ ID NO: 183 - RNA, 19 nt, Synthetic Construct
  source 1..19: mol_type = other RNA; note = modified sense strand of dsRNA; note (original language) = Modified sense strand of dsRNA
  modified_base 1..19: mod_base = OTHER; note = having modifications as shown in Table 3 of the specification
ctgggaccctcaccacgaa

SEQ ID NO: 184 - RNA, 19 nt, Synthetic Construct
  source 1..19: mol_type = other RNA; note = modified sense strand of dsRNA; note (original language) = Modified sense strand of dsRNA
  modified_base 1..19: mod_base = OTHER; note = having modifications as shown in Table 3 of the specification
gccagaagggccaggccaa

SEQ ID NO: 185 - RNA, 19 nt, Synthetic Construct
  source 1..19: mol_type = other RNA; note = modified sense strand of dsRNA; note (original language) = Modified sense strand of dsRNA
  modified_base 1..19: mod_base = OTHER; note = having modifications as shown in Table 3 of the specification
ggccaacgccaccaggata

SEQ ID NO: 186 - RNA, 19 nt, Synthetic Construct
  source 1..19: mol_type = other RNA; note = modified sense strand of dsRNA; note (original language) = Modified sense strand of dsRNA
  modified_base 1..19: mod_base = OTHER; note = having modifications as shown in Table 3 of the specification
aaaacatggccacatccaa

SEQ ID NO: 187 - RNA, 19 nt, Synthetic Construct
  source 1..19: mol_type = other RNA; note = modified sense strand of dsRNA; note (original language) = Modified sense strand of dsRNA
  modified_base 1..19: mod_base = OTHER; note = having modifications as shown in Table 3 of the specification
gaactgctgccatgattta

SEQ ID NO: 188 - RNA, 19 nt, Synthetic Construct
  source 1..19: mol_type = other RNA; note = modified sense strand of dsRNA; note (original language) = Modified sense strand of dsRNA
  modified_base 1..19: mod_base = OTHER; note = having modifications as shown in Table 3 of the specification
ccttctcagtaatgaccca

SEQ ID NO: 189 - RNA, 19 nt, Synthetic Construct
  source 1..19: mol_type = other RNA; note = modified sense strand of dsRNA; note (original language) = Modified sense strand of dsRNA
  modified_base 1..19: mod_base = OTHER; note = having modifications as shown in Table 3 of the specification
catccaactgggaccctca

SEQ ID NO: 190 - RNA, 19 nt, Synthetic Construct
  source 1..19: mol_type = other RNA; note = modified sense strand of dsRNA; note (original language) = Modified sense strand of dsRNA
  modified_base 1..19: mod_base = OTHER; note = having modifications as shown in Table 3 of the specification
ccctcaccacgaatctcaa

SEQ ID NO: 191 - RNA, 19 nt, Synthetic Construct
  source 1..19: mol_type = other RNA; note = modified sense strand of dsRNA; note (original language) = Modified sense strand of dsRNA
  modified_base 1..19: mod_base = OTHER; note = having modifications as shown in Table 3 of the specification
ccgtcacagatgtgagcca

SEQ ID NO: 192 - RNA, 19 nt, Synthetic Construct
  source 1..19: mol_type = other RNA; note = modified sense strand of dsRNA; note (original language) = Modified sense strand of dsRNA
  modified_base 1..19: mod_base = OTHER; note = having modifications as shown in Table 3 of the specification
gaacacacccccttggaaa

SEQ ID NO: 193 - RNA, 19 nt, Synthetic Construct
  source 1..19: mol_type = other RNA; note = modified sense strand of dsRNA; note (original language) = Modified sense strand of dsRNA
  modified_base 1..19: mod_base = OTHER; note = having modifications as shown in Table 3 of the specification
ggcagtggtccgtactcca

SEQ ID NO: 194 - RNA, 19 nt, Synthetic Construct
  source 1..19: mol_type = other RNA; note = modified sense strand of dsRNA; note (original language) = Modified sense strand of dsRNA
  modified_base 1..19: mod_base = OTHER; note = having modifications as shown in Table 3 of the specification
cgaagattgggtccctgga

SEQ ID NO: 195 - RNA, 19 nt, Synthetic Construct
  source 1..19: mol_type = other RNA; note = modified sense strand of dsRNA; note (original language) = Modified sense strand of dsRNA
  modified_base 1..19: mod_base = OTHER; note = having modifications as shown in Table 3 of the specification
ggttggaactgctgccata

SEQ ID NO: 196 - RNA, 19 nt, Synthetic Construct
  source 1..19: mol_type = other RNA; note = modified sense strand of dsRNA; note (original language) = Modified sense strand of dsRNA
  modified_base 1..19: mod_base = OTHER; note = having modifications as shown in Table 3 of the specification
ggtacctactccatactga

SEQ ID NO: 197 - RNA, 19 nt, Synthetic Construct
  source 1..19: mol_type = other RNA; note = modified sense strand of dsRNA; note (original language) = Modified sense strand of dsRNA
  modified_base 1..19: mod_base = OTHER; note = having modifications as shown in Table 3 of the specification
agattgggtccctggacaa

SEQ ID NO: 198 - RNA, 19 nt, Synthetic Construct
  source 1..19: mol_type = other RNA; note = modified sense strand of dsRNA; note (original language) = Modified sense strand of dsRNA
  modified_base 1..19: mod_base = OTHER; note = having modifications as shown in Table 3 of the specification
gggtccctggacaatatca

SEQ ID NO: 199 - RNA, 19 nt, Synthetic Construct
  source 1..19: mol_type = other RNA; note = modified sense strand of dsRNA; note (original language) = Modified sense strand of dsRNA
  modified_base 1..19: mod_base = OTHER; note = having modifications as shown in Table 3 of the specification
agaaggagaggctctgaaa

SEQ ID NO: 200 - RNA, 19 nt, Synthetic Construct
  source 1..19: mol_type = other RNA; note = modified sense strand of dsRNA; note (original language) = Modified sense strand of dsRNA
  modified_base 1..19: mod_base = OTHER; note = having modifications as shown in Table 3 of the specification
ccctgttgtgggggtgtca

SEQ ID NO: 201 - RNA, 19 nt, Synthetic Construct
  source 1..19: mol_type = other RNA; note = modified sense strand of dsRNA; note (original language) = Modified sense strand of dsRNA
  modified_base 1..19: mod_base = OTHER; note = having modifications as shown in Table 3 of the specification
ctgttgtgggggtgtcaca

SEQ ID NO: 202 - RNA, 21 nt, Synthetic Construct
  source 1..21: mol_type = other RNA; note = Unmodified antisense strand of dsRNA
  modified_base 1..21: mod_base = OTHER; note = having modifications as shown in Table 3 of the specification
tctttttatttcctccgccag

SEQ ID NO: 203 - RNA, 21 nt, Synthetic Construct
  source 1..21: mol_type = other RNA; note = modified antisense strand of dsRNA
  modified_base 1..21: mod_base = OTHER; note = having modifications as shown in Table 3 of the specification
tgtcatcgcttccagtcccgt

SEQ ID NO: 204 - RNA, 21 nt, Synthetic Construct
  source 1..21: mol_type = other RNA; note = modified antisense strand of dsRNA
  modified_base 1..21: mod_base = OTHER; note = having modifications as shown in Table 3 of the specification
tttgtcatcgcttccagtccc

SEQ ID NO: 205 - RNA, 21 nt, Synthetic Construct
  source 1..21: mol_type = other RNA; note = modified antisense strand of dsRNA
  modified_base 1..21: mod_base = OTHER; note = having modifications as shown in Table 3 of the specification
ttctttttatttcctccgcca

SEQ ID NO: 206 - RNA, 21 nt, Synthetic Construct
  source 1..21: mol_type = other RNA; note = modified antisense strand of dsRNA
  modified_base 1..21: mod_base = OTHER; note = having modifications as shown in Table 3 of the specification
tgtgggtttcaatctttttat

SEQ ID NO: 207 - RNA, 21 nt, Synthetic Construct
  source 1..21: mol_type = other RNA; note = modified antisense strand of dsRNA
  modified_base 1..21: mod_base = OTHER; note = having modifications as shown in Table 3 of the specification
tcttggtgcatggtgtagccc

SEQ ID NO: 208 - RNA, 21 nt, Synthetic Construct
  source 1..21: mol_type = other RNA; note = modified antisense strand of dsRNA
  modified_base 1..21: mod_base = OTHER; note = having modifications as shown in Table 3 of the specification
tgacattcttcaggtctggca

SEQ ID NO: 209 - RNA, 21 nt, Synthetic Construct
  source 1..21: mol_type = other RNA; note = modified antisense strand of dsRNA
  modified_base 1..21: mod_base = OTHER; note = having modifications as shown in Table 3 of the specification
ttgtacacgatctccgccccg

SEQ ID NO: 210 - RNA, 21 nt, Synthetic Construct
  source 1..21: mol_type = other RNA; note = modified antisense strand of dsRNA
  modified_base 1..21: mod_base = OTHER; note = having modifications as shown in Table 3 of the specification
ttgacattcttcaggtctggc

SEQ ID NO: 211 - RNA, 21 nt, Synthetic Construct
  source 1..21: mol_type = other RNA; note = modified antisense strand of dsRNA
  modified_base 1..21: mod_base = OTHER; note = having modifications as shown in Table 3 of the specification
tggacttgacattcttcaggt

SEQ ID NO: 212 - RNA, 21 nt, Synthetic Construct
  source 1..21: mol_type = other RNA; note = modified antisense strand of dsRNA
  modified_base 1..21: mod_base = OTHER; note = having modifications as shown in Table 3 of the specification
tttgctggaatcctggtggcg

SEQ ID NO: 213 - RNA, 21 nt, Synthetic Construct
  source 1..21: mol_type = other RNA; note = modified antisense strand of dsRNA
  modified_base 1..21: mod_base = OTHER; note = having modifications as shown in Table 3 of the specification
tttggcttttttgtcatcgct

SEQ ID NO: 214 - RNA, 21 nt, Synthetic Construct
  source 1..21: mol_type = other RNA; note = modified antisense strand of dsRNA
  modified_base 1..21: mod_base = OTHER; note = having modifications as shown in Table 3 of the specification
ttgccgtggagacgtgtcccc

SEQ ID NO: 215 - RNA, 21 nt, Synthetic Construct
  source 1..21: mol_type = other RNA; note = modified antisense strand of dsRNA
  modified_base 1..21: mod_base = OTHER; note = having modifications as shown in Table 3 of the specification
ttgatctttcctgtcccccaa

SEQ ID NO: 216 - RNA, 21 nt, Synthetic Construct
  source 1..21: mol_type = other RNA; note = modified antisense strand of dsRNA
  modified_base 1..21: mod_base = OTHER; note = having modifications as shown in Table 3 of the specification
tgcagcttcgtcttccaggct

SEQ ID NO: 217 - RNA, 21 nt, Synthetic Construct
  source 1..21: mol_type = other RNA; note = modified antisense strand of dsRNA
  modified_base 1..21: mod_base = OTHER; note = having modifications as shown in Table 3 of the specification
ttgtcatcgcttccagtcccg

SEQ ID NO: 218 - RNA, 21 nt, Synthetic Construct
  source 1..21: mol_type = other RNA; note = modified antisense strand of dsRNA
  modified_base 1..21: mod_base = OTHER; note = having modifications as shown in Table 3 of the specification
tttttgtcatcgcttccagtc

SEQ ID NO: 219 - RNA, 21 nt, Synthetic Construct
  source 1..21: mol_type = other RNA; note = modified antisense strand of dsRNA
  modified_base 1..21: mod_base = OTHER; note = having modifications as shown in Table 3 of the specification
tttttttgtcatcgcttccag

SEQ ID NO: 220 - RNA, 21 nt, Synthetic Construct
  source 1..21: mol_type = other RNA; note = modified antisense strand of dsRNA
  modified_base 1..21: mod_base = OTHER; note = having modifications as shown in Table 3 of the specification
ttcttcaggtctggcatgggc

SEQ ID NO: 221 - RNA, 21 nt, Synthetic Construct
  source 1..21: mol_type = other RNA; note = modified antisense strand of dsRNA
  modified_base 1..21: mod_base = OTHER; note = having modifications as shown in Table 3 of the specification
ttgtgggtttcaatcttttta

SEQ ID NO: 222 - RNA, 21 nt, Synthetic Construct
  source 1..21: mol_type = other RNA; note = modified antisense strand of dsRNA
  modified_base 1..21: mod_base = OTHER; note = having modifications as shown in Table 3 of the specification
ttggctttggcgttctcgcgg

SEQ ID NO: 223 - RNA, 21 nt, Synthetic Construct
  source 1..21: mol_type = other RNA; note = modified antisense strand of dsRNA
  modified_base 1..21: mod_base = OTHER; note = having modifications as shown in Table 3 of the specification
tccctcttctacatggagggg

SEQ ID NO: 224 - RNA, 21 nt, Synthetic Construct
  source 1..21: mol_type = other RNA; note = modified antisense strand of dsRNA
  modified_base 1..21: mod_base = OTHER; note = having modifications as shown in Table 3 of the specification
ttctccctcttctacatggag

SEQ ID NO: 225 - RNA, 21 nt, Synthetic Construct
  source 1..21: mol_type = other RNA; note = modified antisense strand of dsRNA
  modified_base 1..21: mod_base = OTHER; note = having modifications as shown in Table 3 of the specification
tgtggctccacgaacacacca

SEQ ID NO: 226 - RNA, 21 nt, Synthetic Construct
  source 1..21: mol_type = other RNA; note = modified antisense strand of dsRNA
  modified_base 1..21: mod_base = OTHER; note = having modifications as shown in Table 3 of the specification
taacgggtggacgtctcccaa

SEQ ID NO: 227 - RNA, 21 nt, Synthetic Construct
  source 1..21: mol_type = other RNA; note = modified antisense strand of dsRNA
  modified_base 1..21: mod_base = OTHER; note = having modifications as shown in Table 3 of the specification
ttttgctggaatcctggtggc

SEQ ID NO: 228 - RNA, 21 nt, Synthetic Construct
  source 1..21: mol_type = other RNA; note = modified antisense strand of dsRNA
  modified_base 1..21: mod_base = OTHER; note = having modifications as shown in Table 3 of the specification
ttggaagggacggggtgcggg

SEQ ID NO: 229 - RNA, 21 nt, Synthetic Construct
  source 1..21: mol_type = other RNA; note = modified antisense strand of dsRNA
  modified_base 1..21: mod_base = OTHER; note = having modifications as shown in Table 3 of the specification
tggacgtctcccaagaggcac

SEQ ID NO: 230 - RNA, 21 nt, Synthetic Construct
  source 1..21: mol_type = other RNA; note = modified antisense strand of dsRNA
  modified_base 1..21: mod_base = OTHER; note = having modifications as shown in Table 3 of the specification
tgtgatgaggggtataggcag

SEQ ID NO: 231 - RNA, 21 nt, Synthetic Construct
  source 1..21: mol_type = other RNA; note = modified antisense strand of dsRNA
  modified_base 1..21: mod_base = OTHER; note = having modifications as shown in Table 3 of the specification
tggggtcccactcttgtgcct

SEQ ID NO: 232 - RNA, 21 nt, Synthetic Construct
  source 1..21: mol_type = other RNA; note = modified antisense strand of dsRNA
  modified_base 1..21: mod_base = OTHER; note = having modifications as shown in Table 3 of the specification
ttcgtcttccaggctgggggt

SEQ ID NO: 233 - RNA, 21 nt, Synthetic Construct
  source 1..21: mol_type = other RNA; note = modified antisense strand of dsRNA
  modified_base 1..21: mod_base = OTHER; note = having modifications as shown in Table 3 of the specification
ttggcttttttgtcatcgctt

SEQ ID NO: 234 - RNA, 21 nt, Synthetic Construct
  source 1..21: mol_type = other RNA; note = modified antisense strand of dsRNA
  modified_base 1..21: mod_base = OTHER; note = having modifications as shown in Table 3 of the specification
ttgctggaatcctggtggcgt

SEQ ID NO: 235 - RNA, 21 nt, Synthetic Construct
  source 1..21: mol_type = other RNA; note = modified antisense strand of dsRNA
  modified_base 1..21: mod_base = OTHER; note = having modifications as shown in Table 3 of the specification
ttttatttcctccgccaggga

SEQ ID NO: 236 - RNA, 21 nt, Synthetic Construct
  source 1..21: mol_type = other RNA; note = modified antisense strand of dsRNA
  modified_base 1..21: mod_base = OTHER; note = having modifications as shown in Table 3 of the specification
tttttatttcctccgccaggg

SEQ ID NO: 237 - RNA, 21 nt, Synthetic Construct
  source 1..21: mol_type = other RNA; note = modified antisense strand of dsRNA
  modified_base 1..21: mod_base = OTHER; note = having modifications as shown in Table 3 of the specification
ttctcgcggaaggtcagcttg

SEQ ID NO: 238 - RNA, 21 nt, Synthetic Construct
  source 1..21: mol_type = other RNA; note = modified antisense strand of dsRNA
  modified_base 1..21: mod_base = OTHER; note = having modifications as shown in Table 3 of the specification
ttggcgttctcgcggaaggtc

SEQ ID NO: 239 - RNA, 21 nt, Synthetic Construct
  source 1..21: mol_type = other RNA; note = modified antisense strand of dsRNA
  modified_base 1..21: mod_base = OTHER; note = having modifications as shown in Table 3 of the specification
tttggcgttctcgcggaaggt

SEQ ID NO: 240 - RNA, 21 nt, Synthetic Construct
  source 1..21: mol_type = other RNA; note = modified antisense strand of dsRNA
  modified_base 1..21: mod_base = OTHER; note = having modifications as shown in Table 3 of the specification
tggctttggcgttctcgcgga

SEQ ID NO: 241 - RNA, 21 nt, Synthetic Construct
  source 1..21: mol_type = other RNA; note = modified antisense strand of dsRNA
  modified_base 1..21: mod_base = OTHER; note = having modifications as shown in Table 3 of the specification
tctgcctctgtgacaccccca

SEQ ID NO: 242 - RNA, 21 nt, Synthetic Construct
  source 1..21: mol_type = other RNA; note = modified antisense strand of dsRNA
  modified_base 1..21: mod_base = OTHER; note = having modifications as shown in Table 3 of the specification
ttggaaacgggtggacgtctc

SEQ ID NO: 243 - RNA, 21 nt, Synthetic Construct
  source 1..21: mol_type = other RNA; note = modified antisense strand of dsRNA
  modified_base 1..21: mod_base = OTHER; note = having modifications as shown in Table 3 of the specification
tcacagctgagcagtgccctg

SEQ ID NO: 244 - RNA, 21 nt, Synthetic Construct
  source 1..21: mol_type = other RNA; note = modified antisense strand of dsRNA
  modified_base 1..21: mod_base = OTHER; note = having modifications as shown in Table 3 of the specification
tatgcatgtggagctgagcag

SEQ ID NO: 245 - RNA, 21 nt, Synthetic Construct
  source 1..21: mol_type = other RNA; note = modified antisense strand of dsRNA
  modified_base 1..21: mod_base = OTHER; note = having modifications as shown in Table 3 of the specification
ttccaagggggtgtgttcccc

SEQ ID NO: 246 - RNA, 21 nt, Synthetic Construct
  source 1..21: mol_type = other RNA; note = modified antisense strand of dsRNA
  modified_base 1..21: mod_base = OTHER; note = having modifications as shown in Table 3 of the specification
tggtgcttcaggttctcagtg

SEQ ID NO: 247 - RNA, 21 nt, Synthetic Construct
  source 1..21: mol_type = other RNA; note = modified antisense strand of dsRNA
  modified_base 1..21: mod_base = OTHER; note = having modifications as shown in Table 3 of the specification
taatcatggcagcagttccaa

SEQ ID NO: 248 - RNA, 21 nt, Synthetic Construct
  source 1..21: mol_type = other RNA; note = modified antisense strand of dsRNA
  modified_base 1..21: mod_base = OTHER; note = having modifications as shown in Table 3 of the specification
ttcgtggtgagggtcccagtt

SEQ ID NO: 249 - RNA, 21 nt, Synthetic Construct
  source 1..21: mol_type = other RNA; note = modified antisense strand of dsRNA
  modified_base 1..21: mod_base = OTHER; note = having modifications as shown in Table 3 of the specification
ttggcctggcccttctggcct

SEQ ID NO: 250 - RNA, 21 nt, Synthetic Construct
  source 1..21: mol_type = other RNA; note = modified antisense strand of dsRNA
  modified_base 1..21: mod_base = OTHER; note = having modifications as shown in Table 3 of the specification
tatcctggtggcgttggcctg

SEQ ID NO: 251 - RNA, 21 nt, Synthetic Construct
  source 1..21: mol_type = other RNA; note = modified antisense strand of dsRNA
  modified_base 1..21: mod_base = OTHER; note = having modifications as shown in Table 3 of the specification
ttggatgtggccatgtttttg

SEQ ID NO: 252 - RNA, 21 nt, Synthetic Construct
  source 1..21: mol_type = other RNA; note = modified antisense strand of dsRNA
  modified_base 1..21: mod_base = OTHER; note = having modifications as shown in Table 3 of the specification
taaatcatggcagcagttcca

SEQ ID NO: 253 - RNA, 21 nt, Synthetic Construct
  source 1..21: mol_type = other RNA; note = modified antisense strand of dsRNA
  modified_base 1..21: mod_base = OTHER; note = having modifications as shown in Table 3 of the specification
tgggtcattactgagaagggg

SEQ ID NO: 254 - RNA, 21 nt, Synthetic Construct
  source 1..21: mol_type = other RNA; note = modified antisense strand of dsRNA
  modified_base 1..21: mod_base = OTHER; note = having modifications as shown in Table 3 of the specification
tgagggtcccagttggatgag

SEQ ID NO: 255 - RNA, 21 nt, Synthetic Construct
  source 1..21: mol_type = other RNA; note = modified antisense strand of dsRNA
  modified_base 1..21: mod_base = OTHER; note = having modifications as shown in Table 3 of the specification
ttgagattcgtggtgagggtc

SEQ ID NO: 256 - RNA, 21 nt, Synthetic Construct
  source 1..21: mol_type = other RNA; note = modified antisense strand of dsRNA
  modified_base 1..21: mod_base = OTHER; note = having modifications as shown in Table 3 of the specification
tggctcacatctgtgacggga

SEQ ID NO: 257 - RNA, 21 nt, Synthetic Construct
  source 1..21: mol_type = other RNA; note = modified antisense strand of dsRNA
  modified_base 1..21: mod_base = OTHER; note = having modifications as shown in Table 3 of the specification
tttccaagggggtgtgttccc

SEQ ID NO: 258 - RNA, 21 nt, Synthetic Construct
  source 1..21: mol_type = other RNA; note = modified antisense strand of dsRNA
  modified_base 1..21: mod_base = OTHER; note = having modifications as shown in Table 3 of the specification
tggagtacggaccactgccac

SEQ ID NO: 259 - RNA, 21 nt, Synthetic Construct
  source 1..21: mol_type = other RNA; note = modified antisense strand of dsRNA
  modified_base 1..21: mod_base = OTHER; note = having modifications as shown in Table 3 of the specification
tccagggacccaatcttcgac

SEQ ID NO: 260 - RNA, 21 nt, Synthetic Construct
  source 1..21: mol_type = other RNA; note = modified antisense strand of dsRNA
  modified_base 1..21: mod_base = OTHER; note = having modifications as shown in Table 3 of the specification
tatggcagcagttccaacctt

SEQ ID NO: 261 - RNA, 21 nt, Synthetic Construct
  source 1..21: mol_type = other RNA; note = modified antisense strand of dsRNA
  modified_base 1..21: mod_base = OTHER; note = having modifications as shown in Table 3 of the specification
tcagtatggagtaggtacctc

SEQ ID NO: 262 - RNA, 21 nt, Synthetic Construct
  source 1..21: mol_type = other RNA; note = modified antisense strand of dsRNA
  modified_base 1..21: mod_base = OTHER; note = having modifications as shown in Table 3 of the specification
ttgtccagggacccaatcttc

SEQ ID NO: 263 - RNA, 21 nt, Synthetic Construct
  source 1..21: mol_type = other RNA; note = modified antisense strand of dsRNA
  modified_base 1..21: mod_base = OTHER; note = having modifications as shown in Table 3 of the specification
tgatattgtccagggacccaa

SEQ ID NO: 264 - RNA, 21 nt, Synthetic Construct
  source 1..21: mol_type = other RNA; note = modified antisense strand of dsRNA
  modified_base 1..21: mod_base = OTHER; note = having modifications as shown in Table 3 of the specification
tttcagagcctctccttctcc

SEQ ID NO: 265 - RNA, 21 nt, Synthetic Construct
  source 1..21: mol_type = other RNA; note = modified antisense strand of dsRNA
  modified_base 1..21: mod_base = OTHER; note = having modifications as shown in Table 3 of the specification
tgacacccccacaacagggcc

SEQ ID NO: 266 - RNA, 21 nt, Synthetic Construct
  source 1..21: mol_type = other RNA; note = modified antisense strand of dsRNA
  modified_base 1..21: mod_base = OTHER; note = having modifications as shown in Table 3 of the specification
tgtgacacccccacaacaggg

SEQ ID NO: 267 - RNA, 19 nt, Synthetic Construct
  source 1..19: mol_type = other RNA; note = modified sense strand of dsRNA; note (original language) = Modified sense strand of dsRNA
  modified_base 1..19: mod_base = OTHER; note = having modifications as shown in Table 3 of the specification
gggcggagatcgtgtacaa

SEQ ID NO: 268 - RNA, 19 nt, Synthetic Construct
  source 1..19: mol_type = other RNA; note = modified sense strand of dsRNA; note (original language) = Modified sense strand of dsRNA
  modified_base 1..19: mod_base = OTHER; note = having modifications as shown in Table 3 of the specification
gactggaagcgatgacaaa

SEQ ID NO: 269 - RNA, 19 nt, Synthetic Construct
  source 1..19: mol_type = other RNA; note = modified sense strand of dsRNA; note (original language) = Modified sense strand of dsRNA
  modified_base 1..19: mod_base = OTHER; note = having modifications as shown in Table 3 of the specification
gggactggaagcgatgaca

SEQ ID NO: 270 - RNA, 19 nt, Synthetic Construct
  source 1..19: mol_type = other RNA; note = modified sense strand of dsRNA; note (original language) = Modified sense strand of dsRNA
  modified_base 1..19: mod_base = OTHER; note = having modifications as shown in Table 3 of the specification
ggcggaggaaataaaaaga

SEQ ID NO: 271 - RNA, 19 nt, Synthetic Construct
  source 1..19: mol_type = other RNA; note = modified sense strand of dsRNA; note (original language) = Modified sense strand of dsRNA
  modified_base 1..19: mod_base = OTHER; note = having modifications as shown in Table 3 of the specification
ccagacctgaagaatgtca

SEQ ID NO: 272 - RNA, 19 nt, Synthetic Construct
  source 1..19: mol_type = other RNA; note = modified sense strand of dsRNA; note (original language) = Modified sense strand of dsRNA
  modified_base 1..19: mod_base = OTHER; note = having modifications as shown in Table 3 of the specification
ctgaagaatgtcaagtcca

SEQ ID NO: 273 - RNA, 19 nt, Synthetic Construct
  source 1..19: mol_type = other RNA; note = modified sense strand of dsRNA; note (original language) = Modified sense strand of dsRNA
  modified_base 1..19: mod_base = OTHER; note = having modifications as shown in Table 3 of the specification
gctacaccatgcaccaaga

SEQ ID NO: 274 - RNA, 19 nt, Synthetic Construct
  source 1..19: mol_type = other RNA; note = modified sense strand of dsRNA; note (original language) = Modified sense strand of dsRNA
  modified_base 1..19: mod_base = OTHER; note = having modifications as shown in Table 3 of the specification
aaaaagattgaaacccaca

SEQ ID NO: 275 - RNA, 19 nt, Synthetic Construct
  source 1..19: mol_type = other RNA; note = modified sense strand of dsRNA; note (original language) = Modified sense strand of dsRNA
  modified_base 1..19: mod_base = OTHER; note = having modifications as shown in Table 3 of the specification
cagacctgaagaatgtcaa

SEQ ID NO: 276 - RNA, 19 nt, Synthetic Construct
  source 1..19: mol_type = other RNA; note = modified sense strand of dsRNA; note (original language) = Modified sense strand of dsRNA
  modified_base 1..19: mod_base = OTHER; note = having modifications as shown in Table 3 of the specification
gcggaggaaataaaaagat

SEQ ID NO: 277 - RNA, 21 nt, Synthetic Construct
  source 1..21: mol_type = other RNA; note = modified antisense strand of dsRNA
  modified_base 1..21: mod_base = OTHER; note = having modifications as shown in Table 3 of the specification
ttgtacacgatctccgccccg

SEQ ID NO: 278 - RNA, 21 nt, Synthetic Construct
  source 1..21: mol_type = other RNA; note = modified antisense strand of dsRNA
  modified_base 1..21: mod_base = OTHER; note = having modifications as shown in Table 3 of the specification
tttgtcatcgcttccagtccc

SEQ ID NO: 279 - RNA, 21 nt, Synthetic Construct
  source 1..21: mol_type = other RNA; note = modified antisense strand of dsRNA
  modified_base 1..21: mod_base = OTHER; note = having modifications as shown in Table 3 of the specification
tgtcatcgcttccagtcccgt

SEQ ID NO: 280 - RNA, 21 nt, Synthetic Construct
  source 1..21: mol_type = other RNA; note = modified antisense strand of dsRNA
  modified_base 1..21: mod_base = OTHER; note = having modifications as shown in Table 3 of the specification
tctttttatttcctccgccag

SEQ ID NO: 281 - RNA, 21 nt, Synthetic Construct
  source 1..21: mol_type = other RNA; note = modified antisense strand of dsRNA
  modified_base 1..21: mod_base = OTHER; note = having modifications as shown in Table 3 of the specification
tgacattcttcaggtctggca

SEQ ID NO: 282 - RNA, 21 nt, Synthetic Construct
  source 1..21: mol_type = other RNA; note = modified antisense strand of dsRNA
  modified_base 1..21: mod_base = OTHER; note = having modifications as shown in Table 3 of the specification
tggacttgacattcttcaggt

SEQ ID NO: 283 - RNA, 21 nt, Synthetic Construct
  source 1..21: mol_type = other RNA; note = modified antisense strand of dsRNA
  modified_base 1..21: mod_base = OTHER; note = having modifications as shown in Table 3 of the specification
tcttggtgcatggtgtagccc

SEQ ID NO: 284 - RNA, 21 nt, Synthetic Construct
  source 1..21: mol_type = other RNA; note = modified antisense strand of dsRNA
  modified_base 1..21: mod_base = OTHER; note = having modifications as shown in Table 3 of the specification
tgtgggtttcaatctttttat

SEQ ID NO: 285 - RNA, 21 nt, Synthetic Construct
  source 1..21: mol_type = other RNA; note = modified antisense strand of dsRNA
  modified_base 1..21: mod_base = OTHER; note = having modifications as shown in Table 3 of the specification
ttgacattcttcaggtctggc

SEQ ID NO: 286 - RNA, 21 nt, Synthetic Construct
  source 1..21: mol_type = other RNA; note = modified antisense strand of dsRNA
  modified_base 1..21: mod_base = OTHER; note = having modifications as shown in Table 3 of the specification
atctttttatttcctccgcca

SEQ ID NO: 287 - RNA, 19 nt, Synthetic Construct
  source 1..19: mol_type = other RNA; note = Unmodified sense strand of dsRNA
ggcggagatcgtgtacaac

SEQ ID NO: 288 - RNA, 19 nt, Synthetic Construct
  source 1..19: mol_type = other RNA; note = Unmodified antisense strand of dsRNA
tttgtacacgatctccgcc

SEQ ID NO: 289 - DNA, 22 bp, Synthetic Construct
  source 1..22: PCR_primers = fwd_name: hMAPT, fwd_seq: cctagagcctcacctcctaata,rev_name: hMAPT, rev_seq: caccctcagaattaccgaagaa; mol_type = other DNA
cctagagcctcacctcctaata

SEQ ID NO: 290 - DNA, 22 bp, Synthetic Construct
  source 1..22: PCR_primers = fwd_name: hMAPT, fwd_seq: cctagagcctcacctcctaata,rev_name: hMAPT, rev_seq: caccctcagaattaccgaagaa; mol_type = other DNA
caccctcagaattaccgaagaa

SEQ ID NO: 291 - DNA, 27 bp, Synthetic Construct
  source 1..27: mol_type = other DNA; note = hMAPT-Probe
tgagtttgccatgttgagcaggactat

SEQ ID NO: 292 - DNA, 24 bp, Synthetic Construct
  source 1..24: PCR_primers = fwd_name: hGAPDH, fwd_seq: gaccccttcattgacctcaactac,rev_name: hGAPDH, rev_seq: ttgacggtgccatggaattt; mol_type = other DNA
gaccccttcattgacctcaactac

SEQ ID NO: 293 - DNA, 20 bp, Synthetic Construct
  source 1..20: PCR_primers = fwd_name: hGAPDH, fwd_seq: gaccccttcattgacctcaactac,rev_name: hGAPDH, rev_seq: ttgacggtgccatggaattt; mol_type = other DNA
ttgacggtgccatggaattt

SEQ ID NO: 294 - DNA, 22 bp, Synthetic Construct
  source 1..22: mol_type = other DNA; note = hGAPDH-Probe
ttacatgttccaatatgattcc

SEQ ID NO: 295 - DNA, 22 bp, Synthetic Construct
  source 1..22: PCR_primers = fwd_name: hMAPT, fwd_seq: gacagagtccagtcgaagattg,rev_name: hMAPT, rev_seq: gcgacttgtacacgatctcc; mol_type = other DNA
gacagagtccagtcgaagattg

SEQ ID NO: 296 - DNA, 20 bp, Synthetic Construct
  source 1..20: PCR_primers = fwd_name: hMAPT, fwd_seq: gacagagtccagtcgaagattg,rev_name: hMAPT, rev_seq: gcgacttgtacacgatctcc; mol_type = other DNA
gcgacttgtacacgatctcc

SEQ ID NO: 297 - DNA, 24 bp, Synthetic Construct
  source 1..24: mol_type = other DNA; note = hMAPT-Probe
cgagaacgccaaagccaagacaga

SEQ ID NO: 298 - DNA, 24 bp, Synthetic Construct
  source 1..24: PCR_primers = fwd_name: hGAPDH, fwd_seq: gaccccttcattgacctcaactac,rev_name: hGAPDH, rev_seq: ttgacggtgccatggaattt; mol_type = other DNA
gaccccttcattgacctcaactac

SEQ ID NO: 299 - DNA, 20 bp, Synthetic Construct
  source 1..20: PCR_primers = fwd_name: hGAPDH, fwd_seq: gaccccttcattgacctcaactac,rev_name: hGAPDH, rev_seq: ttgacggtgccatggaattt; mol_type = other DNA
ttgacggtgccatggaattt

SEQ ID NO: 300 - DNA, 22 bp, Synthetic Construct
  source 1..22: mol_type = other DNA; note = hGAPDH-Probe
ttacatgttccaatatgattcc